European Patent Application EP 4 477 655 A1, published December 18, 2024. Title: Phenoxazine derivative and drug delivery system formulation using the same. Applicant: Osaka University. The sequence listing filed with the application follows.

SEQUENCE LISTING (41 sequences)

SEQ ID NO: 1 - DNA, 12 bp, synthetic construct
  misc_feature 1..12: note = ODN 1X
  modified_base 1: mod_base = OTHER; note = G-clamp linker-linked nucleotide
  source 1..12: mol_type = other DNA
gcgttttttgct

SEQ ID NO: 2 - DNA, 12 bp, synthetic construct
  misc_feature 1..12: note = ODN 2X
  modified_base 1: mod_base = OTHER; note = 3 x G-clamp linker-linked nucleotide
  source 1..12: mol_type = other DNA
gcgttttttgct

SEQ ID NO: 3 - DNA, 12 bp, synthetic construct
  misc_feature 1..12: note = ODN No-G-clamp linker-1
  source 1..12: mol_type = other DNA
gcgttttttgct

SEQ ID NO: 4 - DNA, 12 bp, synthetic construct
  misc_feature 1..12: note = ODN No-overhang-1
  source 1..12: mol_type = other DNA
agcaaaaaacgc

SEQ ID NO: 5 - DNA, 16 bp, synthetic construct
  misc_feature 1..16: note = ODN overhang-1
  source 1..16: mol_type = other DNA
agcaaaaaacgcatac

SEQ ID NO: 6 - DNA, 16 bp, synthetic construct
  misc_feature 1..16: note = ODN overhang-2
  source 1..16: mol_type = other DNA
agcaaaaaacgcgtac

SEQ ID NO: 7 - DNA, 16 bp, synthetic construct
  misc_feature 1..16: note = ODN overhang-3
  source 1..16: mol_type = other DNA
agcaaaaaacgctgac

SEQ ID NO: 8 - DNA, 16 bp, synthetic construct
  misc_feature 1..16: note = ODN overhang-4
  source 1..16: mol_type = other DNA
agcaaaaaacgcggtc

SEQ ID NO: 9 - DNA, 16 bp, synthetic construct
  misc_feature 1..16: note = ODN overhang-5
  source 1..16: mol_type = other DNA
agcaaaaaacgctggc

SEQ ID NO: 10 - RNA, 12 nt, synthetic construct
  misc_feature 1..12: note = ON No-overhang-1
  source 1..12: mol_type = other RNA
agcaaaaaacgc

SEQ ID NO: 11 - RNA, 16 nt, synthetic construct
  misc_feature 1..16: note = ON overhang-1
  source 1..16: mol_type = other RNA
agcaaaaaacgcatac

SEQ ID NO: 12 - RNA, 16 nt, synthetic construct
  misc_feature 1..16: note = ON overhang-2
  source 1..16: mol_type = other RNA
agcaaaaaacgcgtac

SEQ ID NO: 13 - RNA, 16 nt, synthetic construct
  misc_feature 1..16: note = ON overhang-3
  source 1..16: mol_type = other RNA
agcaaaaaacgctgac

SEQ ID NO: 14 - RNA, 16 nt, synthetic construct
  misc_feature 1..16: note = ON overhang-4
  source 1..16: mol_type = other RNA
agcaaaaaacgcggtc

SEQ ID NO: 15 - RNA, 16 nt, synthetic construct
  misc_feature 1..16: note = ON overhang-5
  source 1..16: mol_type = other RNA
agcaaaaaacgctggc

SEQ ID NO: 16 - DNA, 12 bp, synthetic construct
  misc_feature 1..12: note = ODN No-G-clamp linker-2
  source 1..12: mol_type = other DNA
gcgttctttgct

SEQ ID NO: 17 - DNA, 12 bp, synthetic construct
  misc_feature 1..12: note = ODN No-overhang-2
  source 1..12: mol_type = other DNA
agcaaagaacgc

SEQ ID NO: 18 - RNA, 12 nt, synthetic construct
  misc_feature 1..12: note = ON No-overhang-2
  source 1..12: mol_type = other RNA
agcaaagaacgc

SEQ ID NO: 19 - DNA, 12 bp, synthetic construct
  misc_feature 1..12: note = ODN mismatch-1
  source 1..12: mol_type = other DNA
agcaaacaacgc

SEQ ID NO: 20 - DNA, 12 bp, synthetic construct
  misc_feature 1..12: note = ODN mismatch-2
  source 1..12: mol_type = other DNA
agcaaaaaacgc

SEQ ID NO: 21 - DNA, 12 bp, synthetic construct
  misc_feature 1..12: note = ODN mismatch-3
  source 1..12: mol_type = other DNA
agcaaataacgc

SEQ ID NO: 22 - RNA, 12 nt, synthetic construct
  misc_feature 1..12: note = ON mismatch-1
  source 1..12: mol_type = other RNA
agcaaacaacgc

SEQ ID NO: 23 - RNA, 12 nt, synthetic construct
  misc_feature 1..12: note = ON mismatch-2
  source 1..12: mol_type = other RNA
agcaaaaaacgc

SEQ ID NO: 24 - RNA, 12 nt, synthetic construct
  misc_feature 1..12: note = ON mismatch-3
  source 1..12: mol_type = other RNA
agcaaataacgc

SEQ ID NO: 25 - DNA, 16 bp, synthetic construct
  misc_feature 1..16: note = GCL(1O)
  modified_base 1: mod_base = OTHER; note = G-clamp linker-linked nucleotide
  modified_base 1: mod_base = OTHER; note = LNA-5-methylcytosine
  modified_base 2..16: mod_base = OTHER; note = phosphorotioated
  modified_base 2: mod_base = OTHER; note = LNA-t
  modified_base 3: mod_base = OTHER; note = LNA-a
  modified_base 14: mod_base = OTHER; note = LNA-t
  modified_base 15: mod_base = OTHER; note = LNA-g
  modified_base 16: mod_base = OTHER; note = LNA-5-methylcytosine
  source 1..16: mol_type = other DNA
ctagttcactgaatgc

SEQ ID NO: 26 - DNA, 16 bp, synthetic construct
  misc_feature 1..16: note = GCL(3O)
  modified_base 1: mod_base = OTHER; note = 3 x G-clamp linker-linked nucleotide
  modified_base 1: mod_base = OTHER; note = LNA-5-methylcytosine
  modified_base 2..16: mod_base = OTHER; note = phosphorotioated
  modified_base 2: mod_base = OTHER; note = LNA-t
  modified_base 3: mod_base = OTHER; note = LNA-a
  modified_base 14: mod_base = OTHER; note = LNA-t
  modified_base 15: mod_base = OTHER; note = LNA-g
  modified_base 16: mod_base = OTHER; note = LNA-5-methylcytosine
  source 1..16: mol_type = other DNA
ctagttcactgaatgc

SEQ ID NO: 27 - DNA, 16 bp, synthetic construct
  misc_feature 1..16: note = GCL(1S)
  modified_base 1: mod_base = OTHER; note = G-clamp linker(PS)-linked nucleotide
  modified_base 1: mod_base = OTHER; note = LNA-5-methylcytosine
  modified_base 2..16: mod_base = OTHER; note = phosphorotioated
  modified_base 2: mod_base = OTHER; note = LNA-t
  modified_base 3: mod_base = OTHER; note = LNA-a
  modified_base 14: mod_base = OTHER; note = LNA-t
  modified_base 15: mod_base = OTHER; note = LNA-g
  modified_base 16: mod_base = OTHER; note = LNA-5-methylcytosine
  source 1..16: mol_type = other DNA
ctagttcactgaatgc

SEQ ID NO: 28 - DNA, 16 bp, synthetic construct
  misc_feature 1..16: note = GCL(3S)
  modified_base 1: mod_base = OTHER; note = 3 x G-clamp linker(PS)-linked nucleotide
  modified_base 1: mod_base = OTHER; note = LNA-5-methylcytosine
  modified_base 2..16: mod_base = OTHER; note = phosphorotioated
  modified_base 2: mod_base = OTHER; note = LNA-t
  modified_base 3: mod_base = OTHER; note = LNA-a
  modified_base 14: mod_base = OTHER; note = LNA-t
  modified_base 15: mod_base = OTHER; note = LNA-g
  modified_base 16: mod_base = OTHER; note = LNA-5-methylcytosine
  source 1..16: mol_type = other DNA
ctagttcactgaatgc

SEQ ID NO: 29 - DNA, 16 bp, synthetic construct
  misc_feature 1..16: note = GCS(1O)
  modified_base 1: mod_base = OTHER; note = G-clamp moiety-linked nucleotide
  modified_base 1: mod_base = OTHER; note = LNA-5-methylcytosine
  modified_base 2..16: mod_base = OTHER; note = phosphorotioated
  modified_base 2: mod_base = OTHER; note = LNA-t
  modified_base 3: mod_base = OTHER; note = LNA-a
  modified_base 14: mod_base = OTHER; note = LNA-t
  modified_base 15: mod_base = OTHER; note = LNA-g
  modified_base 16: mod_base = OTHER; note = LNA-5-methylcytosine
  source 1..16: mol_type = other DNA
ctagttcactgaatgc

SEQ ID NO: 30 - DNA, 16 bp, synthetic construct
  misc_feature 1..16: note = GCS(3O)
  modified_base 1: mod_base = OTHER; note = 3 x G-clamp moiety-linked nucleotide
  modified_base 1: mod_base = OTHER; note = LNA-5-methylcytosine
  modified_base 2..16: mod_base = OTHER; note = phosphorotioated
  modified_base 2: mod_base = OTHER; note = LNA-t
  modified_base 3: mod_base = OTHER; note = LNA-a
  modified_base 14: mod_base = OTHER; note = LNA-t
  modified_base 15: mod_base = OTHER; note = LNA-g
  modified_base 16: mod_base = OTHER; note = LNA-5-methylcytosine
  source 1..16: mol_type = other DNA
ctagttcactgaatgc

SEQ ID NO: 31 - DNA, 16 bp, synthetic construct
  misc_feature 1..16: note = GCS(1S)
  modified_base 1: mod_base = OTHER; note = G-clamp moiety(PS)-linked nucleotide
  modified_base 1: mod_base = OTHER; note = LNA-5-methylcytosine
  modified_base 2..16: mod_base = OTHER; note = phosphorotioated
  modified_base 2: mod_base = OTHER; note = LNA-t
  modified_base 3: mod_base = OTHER; note = LNA-a
  modified_base 14: mod_base = OTHER; note = LNA-t
  modified_base 15: mod_base = OTHER; note = LNA-g
  modified_base 16: mod_base = OTHER; note = LNA-5-methylcytosine
  source 1..16: mol_type = other DNA
ctagttcactgaatgc

SEQ ID NO: 32 - DNA, 16 bp, synthetic construct
  misc_feature 1..16: note = GCS(3S)
  modified_base 1: mod_base = OTHER; note = 3 x G-clamp moiety(PS)-linked nucleotide
  modified_base 1: mod_base = OTHER; note = LNA-5-methylcytosine
  modified_base 2..16: mod_base = OTHER; note = phosphorotioated
  modified_base 2: mod_base = OTHER; note = LNA-t
  modified_base 3: mod_base = OTHER; note = LNA-a
  modified_base 14: mod_base = OTHER; note = LNA-t
  modified_base 15: mod_base = OTHER; note = LNA-g
  modified_base 16: mod_base = OTHER; note = LNA-5-methylcytosine
  source 1..16: mol_type = other DNA
ctagttcactgaatgc

SEQ ID NO: 33 - DNA, 16 bp, synthetic construct
  misc_feature 1..16: note = PXS(1O)
  modified_base 1: mod_base = OTHER; note = dtCO moiety-linked nucleotide
  modified_base 1: mod_base = OTHER; note = LNA-5-methylcytosine
  modified_base 2..16: mod_base = OTHER; note = phosphorotioated
  modified_base 2: mod_base = OTHER; note = LNA-t
  modified_base 3: mod_base = OTHER; note = LNA-a
  modified_base 14: mod_base = OTHER; note = LNA-t
  modified_base 15: mod_base = OTHER; note = LNA-g
  modified_base 16: mod_base = OTHER; note = LNA-5-methylcytosine
  source 1..16: mol_type = other DNA
ctagttcactgaatgc

SEQ ID NO: 34 - DNA, 16 bp, synthetic construct
  misc_feature 1..16: note = PXS(3O)
  modified_base 1: mod_base = OTHER; note = 3 x dtCO moiety-linked nucleotide
  modified_base 1: mod_base = OTHER; note = LNA-5-methylcytosine
  modified_base 2..16: mod_base = OTHER; note = phosphorotioated
  modified_base 2: mod_base = OTHER; note = LNA-t
  modified_base 3: mod_base = OTHER; note = LNA-a
  modified_base 14: mod_base = OTHER; note = LNA-t
  modified_base 15: mod_base = OTHER; note = LNA-g
  modified_base 16: mod_base = OTHER; note = LNA-5-methylcytosine
  source 1..16: mol_type = other DNA
ctagttcactgaatgc

SEQ ID NO: 35 - DNA, 16 bp, synthetic construct
  misc_feature 1..16: note = PXS(1S)
  modified_base 1: mod_base = OTHER; note = dtCO moiety(PS)-linked nucleotide
  modified_base 1: mod_base = OTHER; note = LNA-5-methylcytosine
  modified_base 2..16: mod_base = OTHER; note = phosphorotioated
  modified_base 2: mod_base = OTHER; note = LNA-t
  modified_base 3: mod_base = OTHER; note = LNA-a
  modified_base 14: mod_base = OTHER; note = LNA-t
  modified_base 15: mod_base = OTHER; note = LNA-g
  modified_base 16: mod_base = OTHER; note = LNA-5-methylcytosine
  source 1..16: mol_type = other DNA
ctagttcactgaatgc

SEQ ID NO: 36 - DNA, 16 bp, synthetic construct
  misc_feature 1..16: note = PXS(3S)
  modified_base 1: mod_base = OTHER; note = 3 x dtCO moiety(PS)-linked nucleotide
  modified_base 1: mod_base = OTHER; note = LNA-5-methylcytosine
  modified_base 2..16: mod_base = OTHER; note = phosphorotioated
  modified_base 2: mod_base = OTHER; note = LNA-t
  modified_base 3: mod_base = OTHER; note = LNA-a
  modified_base 14: mod_base = OTHER; note = LNA-t
  modified_base 15: mod_base = OTHER; note = LNA-g
  modified_base 16: mod_base = OTHER; note = LNA-5-methylcytosine
  source 1..16: mol_type = other DNA
ctagttcactgaatgc

SEQ ID NO: 37 - RNA, 20 nt, Mus musculus
  source 1..20: mol_type = transcribed RNA
gcattcagtgaactaggaag

SEQ ID NO: 38 - DNA, 20 bp, synthetic construct
  misc_feature 1..20: note = PCR Primer(mMalat1_F4)
  source 1..20: mol_type = other DNA
acattccttgaggtcggcaa

SEQ ID NO: 39 - DNA, 20 bp, synthetic construct
  misc_feature 1..20: note = PCR Primer(mMalat1_R4)
  source 1..20: mol_type = other DNA
cacccgcaaaggcctacata

SEQ ID NO: 40 - DNA, 19 bp, synthetic construct
  misc_feature 1..19: note = PCR Primer(mGapdh_F3)
  source 1..19: mol_type = other DNA
tcaccaccatggagaaggc

SEQ ID NO: 41 - DNA, 20 bp, synthetic construct
  misc_feature 1..20: note = PCR Primer(mGapdh_R3)
  source 1..20: mol_type = other DNA
gctaagcagttggtggtgca